European Patent Application EP 4 119 578 A1, published January 18, 2023. Title: ANTI-BCMA-BINDING DOMAINS, FUSION PROTEINS COMPRISING THEREOF, AND COMPOSITIONS COMPRISING THEREOF. Applicant: CUROCELL INC. Ewha University-Industry Collaboration Foundation. The sequence listing filed with the application follows.

SEQUENCE LISTING (15 sequences)

SEQ ID NO: 1 - protein, 5 aa, Artificial Sequence
  VH-CDR1
DYYMS

SEQ ID NO: 2 - protein, 17 aa, Artificial Sequence
  VH-CDR2
AISHSSGNTYYADSVKG

SEQ ID NO: 3 - protein, 9 aa, Artificial Sequence
  VH-CDR3
AKNNWGFDY

SEQ ID NO: 4 - protein, 13 aa, Artificial Sequence
  VL-CDR1
TGSSSNIGSNDVT

SEQ ID NO: 5 - protein, 7 aa, Artificial Sequence
  VL-CDR2
SDSKRPS

SEQ ID NO: 6 - protein, 11 aa, Artificial Sequence
  VL-CDR3
AAWDASLSGYV

SEQ ID NO: 7 - protein, 116 aa, Artificial Sequence
  VH
EVQLLESGGGLVQPGGSLRLSCAASGFTFSDYYMSWVRLAPGKGLEWVSAISHSSGNTYYADSVKGRFTISRDNSKNTLYLQMNSLRAEDTAVYYCAKNNWGFDYWGQGTLVTVSS

SEQ ID NO: 8 - protein, 110 aa, Artificial Sequence
  VL
QSVLTQPPSASGTPGQRVTISCTGSSSNIGSNDVTWYQQLPGTAPKLLIYSDSKRPSGVPDRFSGSKSGTSASLAISGLRSEDEADYYCAAWDASLSGYVFGGGTKLTVL

SEQ ID NO: 9 - protein, 241 aa, Artificial Sequence
  scFv
EVQLLESGGGLVQPGGSLRLSCAASGFTFSDYYMSWVRLAPGKGLEWVSAISHSSGNTYYADSVKGRFTISRDNSKNTLYLQMNSLRAEDTAVYYCAKNNWGFDYWGQGTLVTVSSGGGGSGGGGSGGGGSQSVLTQPPSASGTPGQRVTISCTGSSSNIGSNDVTWYQQLPGTAPKLLIYSDSKRPSGVPDRFSGSKSGTSASLAISGLRSEDEADYYCAAWDASLSGYVFGGGTKLTVL

SEQ ID NO: 10 - protein, 112 aa, Artificial Sequence
  CD3zeta signaling domain
RVKFSRSADAPAYQQGQNQLYNELNLGRREEYDVLDKRRGRDPEMGGKPRRKNPQEGLYNELQKDKMAEAYSEIGMKGERRRGKGHDGLYQGLSTATKDTYDALHMQALPPR

SEQ ID NO: 11 - protein, 42 aa, Artificial Sequence
  41BB signaling domain
KRGRKKLLYIFKQPFMRPVQTTQEEDGCSCRFPEEEEGGCEL

SEQ ID NO: 12 - protein, 24 aa, Artificial Sequence
  transmembrane domain
IYIWAPLAGTCGVLLLSLVITLYC

SEQ ID NO: 13 - protein, 45 aa, Artificial Sequence
  hinge domain
TTTPAPRPPTPAPTIASQPLSLRPEACRPAAGGAVHTRGLDFACD

SEQ ID NO: 14 - protein, 21 aa, Artificial Sequence
  signal peptide
MALPVTALLLPLALLLHAARP

SEQ ID NO: 15 - protein, 485 aa, Artificial Sequence
  a-BCMA CAR
MALPVTALLLPLALLLHAARPEVQLLESGGGLVQPGGSLRLSCAASGFTFSDYYMSWVRLAPGKGLEWVSAISHSSGNTYYADSVKGRFTISRDNSKNTLYLQMNSLRAEDTAVYYCAKNNWGFDYWGQGTLVTVSSGGGGSGGGGSGGGGSQSVLTQPPSASGTPGQRVTISCTGSSSNIGSNDVTWYQQLPGTAPKLLIYSDSKRPSGVPDRFSGSKSGTSASLAISGLRSEDEADYYCAAWDASLSGYVFGGGTKLTVLTTTPAPRPPTPAPTIASQPLSLRPEACRPAAGGAVHTRGLDFACDIYIWAPLAGTCGVLLLSLVITLYCKRGRKKLLYIFKQPFMRPVQTTQEEDGCSCRFPEEEEGGCELRVKFSRSADAPAYKQGQNQLYNELNLGRREEYDVLDKRRGRDPEMGGKPRRKNPQEGLYNELQKDKMAEAYSEIGMKGERRRGKGHDGLYQGLSTATKDTYDALHMQALPPR